European Patent Application EP 4 306 128 A2, published January 17, 2024. Title: SUBCUTANEOUS DOSAGE AND ADMINISTRATION OF ANTI-C5 ANTIBODIES FOR TREATMENT OF PAROXYSMAL NOCTURNAL HEMOGLOBINURIA (PNH). Applicant: ALEXION PHARMACEUTICALS, INC. Application EP 23200753.4, filed October 30, 2019. The sequence listing filed with the application follows.

SEQUENCE LISTING (50 sequences)

SEQ ID NO: 1 - protein, 10 aa, synthetic construct
  REGION 1..10: note = synthetic peptide
GYIFSNYWIQ

SEQ ID NO: 2 - protein, 17 aa, synthetic construct
  REGION 1..17: note = synthetic peptide
EILPGSGSTEYTENFKD

SEQ ID NO: 3 - protein, 13 aa, synthetic construct
  REGION 1..13: note = synthetic peptide
YFFGSSPNWYFDV

SEQ ID NO: 4 - protein, 11 aa, synthetic construct
  REGION 1..11: note = synthetic peptide
GASENIYGALN

SEQ ID NO: 5 - protein, 7 aa, synthetic construct
  REGION 1..7: note = synthetic peptide
GATNLAD

SEQ ID NO: 6 - protein, 9 aa, synthetic construct
  REGION 1..9: note = synthetic peptide
QNVLNTPLT

SEQ ID NO: 7 - protein, 122 aa, synthetic construct [sequence omitted]

SEQ ID NO: 8 - protein, 107 aa, synthetic construct [sequence omitted]

SEQ ID NO: 9 - protein, 326 aa, synthetic construct
  REGION 1..326: note = synthetic polypeptide
ASTKGPSVFPLAPCSRSTSESTAALGCLVKDYFPEPVTVSWNSGALTSGVHTFPAVLQSSGLYSLSSVVTVPSSNFGTQTYTCNVDHKPSNTKVDKTVERKCCVECPPCPAPPVAGPSVFLFPPKPKDTLMISRTPEVTCVVVDVSQEDPEVQFNWYVDGVEVHNAKTKPREEQFNSTYRVVSVLTVLHQDWLNGKEYKCKVSNKGLPSSIEKTISKAKGQPREPQVYTLPPSQEEMTKNQVSLTCLVKGFYPSDIAVEWESNGQPENNYKTTPPVLDSDGSFFLYSRLTVDKSRWQEGNVFSCSVMHEALHNHYTQKSLSLSLGK

SEQ ID NO: 10 - protein, 448 aa, synthetic construct
  REGION 1..448: note = synthetic polypeptide
QVQLVQSGAEVKKPGASVKVSCKASGYIFSNYWIQWVRQAPGQGLEWMGEILPGSGSTEYTENFKDRVTMTRDTSTSTVYMELSSLRSEDTAVYYCARYFFGSSPNWYFDVWGQGTLVTVSSASTKGPSVFPLAPCSRSTSESTAALGCLVKDYFPEPVTVSWNSGALTSGVHTFPAVLQSSGLYSLSSVVTVPSSNFGTQTYTCNVDHKPSNTKVDKTVERKCCVECPPCPAPPVAGPSVFLFPPKPKDTLMISRTPEVTCVVVDVSQEDPEVQFNWYVDGVEVHNAKTKPREEQFNSTYRVVSVLTVLHQDWLNGKEYKCKVSNKGLPSSIEKTISKAKGQPREPQVYTLPPSQEEMTKNQVSLTCLVKGFYPSDIAVEWESNGQPENNYKTTPPVLDSDGSFFLYSRLTVDKSRWQEGNVFSCSVMHEALHNHYTQKSLSLSLGK

SEQ ID NO: 11 - protein, 214 aa, synthetic construct [sequence omitted]

SEQ ID NO: 12 - protein, 122 aa, synthetic construct [sequence omitted]

SEQ ID NO: 13 - protein, 326 aa, synthetic construct
  REGION 1..326: note = synthetic polypeptide
ASTKGPSVFPLAPCSRSTSESTAALGCLVKDYFPEPVTVSWNSGALTSGVHTFPAVLQSSGLYSLSSVVTVPSSNFGTQTYTCNVDHKPSNTKVDKTVERKCCVECPPCPAPPVAGPSVFLFPPKPKDTLMISRTPEVTCVVVDVSQEDPEVQFNWYVDGVEVHNAKTKPREEQFNSTYRVVSVLTVLHQDWLNGKEYKCKVSNKGLPSSIEKTISKAKGQPREPQVYTLPPSQEEMTKNQVSLTCLVKGFYPSDIAVEWESNGQPENNYKTTPPVLDSDGSFFLYSRLTVDKSRWQEGNVFSCSVLHEALHSHYTQKSLSLSLGK

SEQ ID NO: 14 - protein, 448 aa, synthetic construct
  REGION 1..448: note = synthetic polypeptide
QVQLVQSGAEVKKPGASVKVSCKASGHIFSNYWIQWVRQAPGQGLEWMGEILPGSGHTEYTENFKDRVTMTRDTSTSTVYMELSSLRSEDTAVYYCARYFFGSSPNWYFDVWGQGTLVTVSSASTKGPSVFPLAPCSRSTSESTAALGCLVKDYFPEPVTVSWNSGALTSGVHTFPAVLQSSGLYSLSSVVTVPSSNFGTQTYTCNVDHKPSNTKVDKTVERKCCVECPPCPAPPVAGPSVFLFPPKPKDTLMISRTPEVTCVVVDVSQEDPEVQFNWYVDGVEVHNAKTKPREEQFNSTYRVVSVLTVLHQDWLNGKEYKCKVSNKGLPSSIEKTISKAKGQPREPQVYTLPPSQEEMTKNQVSLTCLVKGFYPSDIAVEWESNGQPENNYKTTPPVLDSDGSFFLYSRLTVDKSRWQEGNVFSCSVLHEALHSHYTQKSLSLSLGK

SEQ ID NO: 15 - protein, 326 aa, synthetic construct
  REGION 1..326: note = synthetic polypeptide
ASTKGPSVFPLAPCSRSTSESTAALGCLVKDYFPEPVTVSWNSGALTSGVHTFPAVLQSSGLYSLSSVVTVTSSNFGTQTYTCNVDHKPSNTKVDKTVERKCCVECPPCPAPPVAGPSVFLFPPKPKDTLYITREPEVTCVVVDVSHEDPEVQFNWYVDGMEVHNAKTKPREEQFNSTFRVVSVLTVVHQDWLNGKEYKCKVSNKGLPAPIEKTISKTKGQPREPQVYTLPPSREEMTKNQVSLTCLVKGFYPSDIAVEWESNGQPENNYKTTPPMLDSDGSFFLYSKLTVDKSRWQQGNVFSCSVMHEALHNHYTQKSLSLSPGK

SEQ ID NO: 16 - protein, 448 aa, synthetic construct
  REGION 1..448: note = synthetic polypeptide
QVQLVQSGAEVKKPGASVKVSCKASGYIFSNYWIQWVRQAPGQGLEWMGEILPGSGSTEYTENFKDRVTMTRDTSTSTVYMELSSLRSEDTAVYYCARYFFGSSPNWYFDVWGQGTLVTVSSASTKGPSVFPLAPCSRSTSESTAALGCLVKDYFPEPVTVSWNSGALTSGVHTFPAVLQSSGLYSLSSVVTVTSSNFGTQTYTCNVDHKPSNTKVDKTVERKCCVECPPCPAPPVAGPSVFLFPPKPKDTLYITREPEVTCVVVDVSHEDPEVQFNWYVDGMEVHNAKTKPREEQFNSTFRVVSVLTVVHQDWLNGKEYKCKVSNKGLPAPIEKTISKTKGQPREPQVYTLPPSREEMTKNQVSLTCLVKGFYPSDIAVEWESNGQPENNYKTTPPMLDSDGSFFLYSKLTVDKSRWQQGNVFSCSVMHEALHNHYTQKSLSLSPGK

SEQ ID NO: 17 - protein, 11 aa, synthetic construct
  REGION 1..11: note = synthetic peptide
GASENIYHALN

SEQ ID NO: 18 - protein, 17 aa, synthetic construct
  REGION 1..17: note = synthetic peptide
EILPGSGHTEYTENFKD

SEQ ID NO: 19 - protein, 10 aa, synthetic construct
  REGION 1..10: note = synthetic peptide
GHIFSNYWIQ

SEQ ID NO: 20 - protein, 448 aa, synthetic construct
  REGION 1..448: note = synthetic polypeptide
QVQLVQSGAEVKKPGASVKVSCKASGHIFSNYWIQWVRQAPGQGLEWMGEILPGSGHTEYTENFKDRVTMTRDTSTSTVYMELSSLRSEDTAVYYCARYFFGSSPNWYFDVWGQGTLVTVSSASTKGPSVFPLAPCSRSTSESTAALGCLVKDYFPEPVTVSWNSGALTSGVHTFPAVLQSSGLYSLSSVVTVPSSNFGTQTYTCNVDHKPSNTKVDKTVERKCCVECPPCPAPPVAGPSVFLFPPKPKDTLMISRTPEVTCVVVDVSQEDPEVQFNWYVDGVEVHNAKTKPREEQFNSTYRVVSVLTVLHQDWLNGKEYKCKVSNKGLPSSIEKTISKAKGQPREPQVYTLPPSQEEMTKNQVSLTCLVKGFYPSDIAVEWESNGQPENNYKTTPPVLDSDGSFFLYSRLTVDKSRWQEGNVFSCSVMHEALHNHYTQKSLSLSLGK

SEQ ID NO: 21 - protein, 5 aa, synthetic construct
  REGION 1..5: note = synthetic peptide
SYAIS

SEQ ID NO: 22 - protein, 17 aa, synthetic construct
  REGION 1..17: note = synthetic peptide
GIGPFFGTANYAQKFQG

SEQ ID NO: 23 - protein, 7 aa, synthetic construct
  REGION 1..7: note = synthetic peptide
DTPYFDY

SEQ ID NO: 24 - protein, 11 aa, synthetic construct
  REGION 1..11: note = synthetic peptide
SGDSIPNYYVY

SEQ ID NO: 25 - protein, 7 aa, synthetic construct
  REGION 1..7: note = synthetic peptide
DDSNRPS

SEQ ID NO: 26 - protein, 11 aa, synthetic construct
  REGION 1..11: note = synthetic peptide
QSFDSSLNAEV

SEQ ID NO: 27 - protein, 116 aa, synthetic construct
  REGION 1..116: note = synthetic polypeptide
QVQLVQSGAEVKKPGSSVKVSCKASGGTFSSYAISVWRQAPGQGLEWMGGIGPFFGTANYAQKFQGRVTITADESTSTAYMELSSLRSEDTAVYYCARDTPYFDYWGQGTLVTVSS

SEQ ID NO: 28 - protein, 108 aa, synthetic construct
  REGION 1..108: note = synthetic polypeptide
DIELTQPPSVSVAPGQTARISCSGDSIPNYYVYWYQQKPGQAPVLVIYDDSNRPSGIPERFSGSNSGNTATLTISGTQAEDEADYYCQSFDSSLNAEVFGGGTKLTVL

SEQ ID NO: 29 - protein, 4 aa, synthetic construct
  REGION 1..4: note = synthetic peptide
NYIS

SEQ ID NO: 30 - protein, 17 aa, synthetic construct
  REGION 1..17: note = synthetic peptide
IIDPDDSYTEYSPSFQG

SEQ ID NO: 31 - protein, 8 aa, synthetic construct
  REGION 1..8: note = synthetic peptide
YEYGGFDI

SEQ ID NO: 32 - protein, 11 aa, synthetic construct
  REGION 1..11: note = synthetic peptide
SGDNIGNSYVH

SEQ ID NO: 33 - protein, 7 aa, synthetic construct
  REGION 1..7: note = synthetic peptide
KDNDRPS

SEQ ID NO: 34 - protein, 9 aa, synthetic construct
  REGION 1..9: note = synthetic peptide
GTYDIESYV

SEQ ID NO: 35 - protein, 116 aa, synthetic construct
  REGION 1..116: note = synthetic polypeptide
EVQLVQSGAEVKKPGESLKISCKGSGYSFTNYISWVRQMPGKGLEWMGIIDPDDSYTEYSPSFQGQVTISADKSISTAYLQWSSLKASDTAMYYCARYEYGGFDIWGQGTLVTVSS

SEQ ID NO: 36 - protein, 106 aa, synthetic construct
  REGION 1..106: note = synthetic polypeptide
SYELTQPPSVSVAPGQTARISCSGDNIGNSYVHWYQQKPGQAPVLVIYKDNDRPSGIPERFSGSNSGNTATLTISGTQAEDEADYYCGTYDIESYVFGGGTKLTVL

SEQ ID NO: 37 - protein, 6 aa, synthetic construct
  REGION 1..6: note = synthetic peptide
SSYYVA

SEQ ID NO: 38 - protein, 17 aa, synthetic construct
  REGION 1..17: note = synthetic peptide
AIYTGSGATYKASWAKG

SEQ ID NO: 39 - protein, 13 aa, synthetic construct
  REGION 1..13: note = synthetic peptide
DGGYDYPTHAMHY

SEQ ID NO: 40 - protein, 11 aa, synthetic construct
  REGION 1..11: note = synthetic peptide
QASQNIGSSLA

SEQ ID NO: 41 - protein, 7 aa, synthetic construct
  REGION 1..7: note = synthetic peptide
GASKTHS

SEQ ID NO: 42 - protein, 12 aa, synthetic construct
  REGION 1..12: note = synthetic peptide
QSTKVGSSYGNH

SEQ ID NO: 43 - protein, 123 aa, synthetic construct
  REGION 1..123: note = synthetic polypeptide
QVQLVESGGGLVQPGGSLRLSCAASGFTSHSSYYVAWVRQAPGKGLEWVGAIYTGSGATYKASWAKGRFTISKDTSKNQVVLTMTNMDPVDTATYYCASDGGYDYPTHAMHYWGQGTLVTVSS

SEQ ID NO: 44 - protein, 110 aa, synthetic construct
  REGION 1..110: note = synthetic polypeptide
DVVMTQSPSSLSASVGDRVTITCQASQNIGSSLAWYQQKPGQAPRLLIYGASKTHSGVPSRFSGSGSGTDFTLTISSLQPEDVATYYCQSTKVGSSYGNHFGGGTKVEIK

SEQ ID NO: 45 - protein, 451 aa, synthetic construct
  REGION 1..451: note = synthetic polypeptide
QVQLVESGGGLVQPGRSLRLSCAASGFTVHSSYYMAWVRQAPGKGLEWVGAIFTGSGAEYKAEWAKGRVTISKDTSKNQVVLTMTNMDPVDTATYYCASDAGYDYPTHAMHYWGQGTLVTVSSASTKGPSVFPLAPSSKSTSGGTAALGCLVKDYFPEPVTVSWNSGALTSGVHTFPAVLQSSGLYSLSSVVTVPSSSLGTQTYICNVNHKPSNTKVDKKVEPKSCDKTHTCPPCPAPELRRGPKVFLFPPKPKDTLMISRTPEVTCVVVDVSHEDPEVKFNWYVDGVEVHNAKTKPREEQYNSTYRVVSVLTVLHQDWLNGKEYKCKVSNKGLPSSIEKTISKAKGQPREPQVYTLPPSREEMTKNQVSLTCLVKGFYPSDIAVEWESNGQPENNYKTTPPVLDSDGSFFLYSKLTVDKSRWQQGNVFSCSVLHEALHAHYTRKELSLSP

SEQ ID NO: 46 - protein, 217 aa, synthetic construct
  REGION 1..217: note = synthetic polypeptide
DIQMTQSPSSLSASVGDRVTITCRASQGISSSLAWYQQKPGKAPKLLIYGASETESGVPSRFSGSGSGTDFTLTISSLQPEDFATYYCQNTKVGSSYGNTFGGGTKVEIKRTVAAPSVFIFPPSDEQLKSGTASVVCLLNNFYPREAKVQWKVDNALQSGNSQESVTEQDSKDSTYSLSSTLTLSKADYEKHKVYACEVTHQGLSSPVTKSFNRGEC

SEQ ID NO: 47 - protein, 120 aa, synthetic construct
  REGION 1..120: note = synthetic polypeptide
QVQLQESGPGLVKPSETLSLTCTVSGDSVSSSYWTWIRQPPGKGLEWIGYIYYSGSSNYNPSLKSRATISVDTSKNQFSLKLSSVTAADTAVYYCAREGNVDTTMIFDYWGQGTLVTVSS

SEQ ID NO: 48 - protein, 107 aa, synthetic construct
  REGION 1..107: note = synthetic polypeptide
AIQMTQSPSSLSASVGDRVTITCRASQGIRNDLGWYQQKPGKAPKLLIYAASSLQSGVPSRFAGRGSGTDFTLTISSLQPEDFATYYCLQDFNYPWTFGQGTKVEIK

SEQ ID NO: 49 - protein, 447 aa, synthetic construct
  REGION 1..447: note = synthetic polypeptide
QVQLQESGPGLVKPSETLSLTCTVSGDSVSSSYWTWIRQPPGKGLEWIGYIYYSGSSNYNPSLKSRATISVDTSKNQFSLKLSSVTAADTAVYYCAREGNVDTTMIFDYWGQGTLVTVSSASTKGPSVFPLAPCSRSTSESTAALGCLVKDYFPEPVTVSWNSGALTSGVHTFPAVLQSSGLYSLSSVVTVPSSSLGTKTYTCNVDHKPSNTKVDKRVESKYGPPCPPCPAPEFLGGPSVFLFPPKPKDTLMISRTPEVTCVVVDVSQEDPEVQFNWYVDGVEVHNAKTKPREEQFNSTYRVVSVLTVLHQDWLNGKEYKCKVSNKGLPSSIEKTISKAKGQPREPQVYTLPPSQEEMTKNQVSLTCLVKGFYPSDIAVEWESNGQPENNYKTTPPVLDSDGSFFLYSRLTVDKSRWQEGNVFSCSVMHEALHNHYTQKSLSLSLGK

SEQ ID NO: 50 - protein, 214 aa, synthetic construct
  REGION 1..214: note = synthetic polypeptide
AIQMTQSPSSLSASVGDRVTITCRASQGIRNDLGWYQQKPGKAPKLLIYAASSLQSGVPSRFAGRGSGTDFTLTISSLQPEDFATYYCLQDFNYPWTFGQGTKVEIKRTVAAPSVFIFPPSDEQLKSGTASVVCLLNNFYPREAKVQWKVDNALQSGNSQESVTEQDSKDSTYSLSSTLTLSKADYEKHKVYACEVTHQGLSSPVTKSFNRGEC